European Patent Specification EP 3 701 001 B1, published June 10, 2026. Title: COMPOSITIONS COMPRISING POLYPEPTIDES HAVING MANNANASE ACTIVITY. Applicant: Novozymes A/S. The sequence listing filed with the application follows.

SEQUENCE LISTING (23 sequences)

SEQ ID NO: 1 - protein, 326 aa, Bacillus bogoriensis
  SIGNAL (1)..(28)
  mat_peptide (29)..(326)
MKQQKRLYARLLTLLFALIFLLPHSAAAANSGFYVSGTTLYDANGNPFVMRGINHGHAWYKDQATTAIEGIANTGANTVRIVLSDGGQWTKDDIHTVRNLISLAEDNHLVAVLEVHDATGYDSIASLNRAVDYWIEMRSALIGKEDTVIINIANEWFGSWEGDAWADGYKQAIPRLRNAGLNHTLMVDAAGWGQFPQSIHDYGREVFNADPQRNTMFSIHMYEYAGGNASQVRTNIDRVLNQDLALVIGEFGHRHTNGDVDEATIMSYSEQRGVGWLAWSWKGNGPEWEYLDLSNDWAGNNLTAWGNTIVNGPYGLRETSRLSTVF

SEQ ID NO: 2 - protein, 298 aa, Bacillus bogoriensis
ANSGFYVSGTTLYDANGNPFVMRGINHGHAWYKDQATTAIEGIANTGANTVRIVLSDGGQWTKDDIHTVRNLISLAEDNHLVAVLEVHDATGYDSIASLNRAVDYWIEMRSALIGKEDTVIINIANEWFGSWEGDAWADGYKQAIPRLRNAGLNHTLMVDAAGWGQFPQSIHDYGREVFNADPQRNTMFSIHMYEYAGGNASQVRTNIDRVLNQDLALVIGEFGHRHTNGDVDEATIMSYSEQRGVGWLAWSWKGNGPEWEYLDLSNDWAGNNLTAWGNTIVNGPYGLRETSRLSTVF

SEQ ID NO: 3 - protein, 330 aa, Paenibacillus woosongensis
IRTGTLNNPEATAEARALMNYLLSQYGQKIISGQQTLEDVEWIKQQTGKYPAIFSTDLMDYSPSRVDHGASSTEVEKMIEWYKRGGIVSLCWHWNAPKGIGGNEPGNEWWRGFYTEFTTFDVEYALNHPDSEDYQLLIRDIDAIAVQLKRLQEANVPVLWRPLHEAEGTWFWWGAKGPEPAKQLYRLMYDRLTNDHKLNNLIWVWNSEKKDWYPGDDVVDMVSVDIYNPAGDYNPSIAKYEALVSLADNKKMAALAENGPIPDPDALQEYGADWSFFSTWTGDYIRDGKTNTIEHLKKVYQHDYVITLDELPADCTPILMIRQRMVNQQG

SEQ ID NO: 4 - protein, 312 aa, Paenibacillus illinoisensis
ASPQAKALMKFMTNQYGKKIISGQQTLEDAAWIYQQTGKYPALVSSDLMDYSPSRVENGSTSNEVEKMMEWYKRGGIVSLSWHWNAPKGIGSNEPGHEWWRGFNTEFTTFDVEYALNHPESEDYKLLIRDIDAIATQLKRLQEHHIPVLWRPLHEAEGGWFWWGAKGPEPAKKLYRLMYERLTEKHGLNNLIWVWNSVKEEWYPGDDVVDMVSVDIYNPPGDYSPNIAKYDELLFLSKHKKLVALAENGPIPDPDLLQTYGAHWSYFNTWTGDVLRDGKTNTKEHLKKVYNHDNVITLDELPKGLYDSPRWK

SEQ ID NO: 5 - protein, 699 aa, Neobulgaria sp.
TVFEAEKGTLAGGLTIATDVTGYTGTGYVTNFADAAALLTFTVNGLTAGSYDLTLTYSAQYGDKFTTVSVNGASGIEVAITNVTTATWTTATIGTFTLTAGDNTVSCADDWGWYLIDSLTVIPTPAKPITIVDVSNGATAQAEDGILTGTTVGTTTAGYTGTGYVTGFTATGTQVTINLSSTKQALYDVVVRYAAIYGQKYTTMQLNGVGGSEILLLDTTTATSPWANATAGQVLLASGNNTLTFMNDWGWYFIDAVYVTPSPAPAPHKVTNALVDAKALASTHALFNTLLAKYGSGDIFSGQADPTGVTWIESNLGTTKTPAIIGLDMIEYSPTRVLYGSTSTAVEDAIAFDKRGGMVAFQWHWNAPADLINNDTVPWWKGFYSYGTTFNLTAALANPSGSDYALLISDMDAIAVQLLRLQAAGVPVLWRPLHEADGTWFWWGNFGAASCVSLYRIMYDRYTNYHGLHNLIWVWNSVTPSWYPGADVVDILGYDSYPAVGDHGPVSSQYNALITLGGDTKLVTLPEVGNIPDPAILKLYHADWSYFVTWNQDYILTDTYNPLAFKQQVYNDPTVLKLTDLGNWKGAATSTIVSSTSKVSTTTSSLITSTTKKTSSSTVVSTTSSTVKTTSTTSKVSSSTTKVSSTTKVTTTSTTTSAVATATAGHWGQCGGTGWTGPTVCASGFTCTAVSPPYYYQCL

SEQ ID NO: 6 - protein, 452 aa, Preussia aemulans
QTVIYQAEQAKLSGVTVEFSIIKQVVGTGYVEGFDESTDSITFTVESTTAALYDLALTYNGPYGDKYTNVVLNNAAGSQVSLPATTAWTTVPAGQVLLNAGANTIQIQNNWGWYLVDSISLKPAATRGAHQITTKPVNKNANSDAKALLKYLGSIYGKKILSGQQDLSSLDWVTKNVGKTPAVLGLDTMDYSESRKSRGAVSTDVDKAIAFAKKGGIVTFCWHWGAPTGLFDSAAQPWYRGFYTDATDFNIETALKDTTNANYTLLMKDIDTIAVQLKKLQDAGVPVIWRPLHEAEGGWFWWGAKGPEPAKKLWKIMYDRLTNQHGLNNLVWTWNSVAPNWYPGDDTVDIVSADTYSQGDHGPISATYNNLLALTNDTKIIAAAEIGSVMEPAQLQAYQADWVYFCVWSGEFIDGGVWNSLDFLKKVYNDPYVLTLDEIQGWKTARGKPRVS

SEQ ID NO: 7 - protein, 312 aa, Yunnania penicillata
APSTTPVNEKATDAAKNLLSYLVEQAANGVTLSGQQDLESAQWVSDNVGKWPAILGIDFMDYSPSRVEYGAVGSTVPDAISYDSDGGIVTFCWHWGSPSGTYNTTDQPWWSNFYTEATAFDIAAAMDDPDSADYNLLVRDIDAISELLLQLQDLDIPILWRPLHEAEGGWFWWGAKGPEACIALYRLMFDRMTNHHGLNNLLWVWNSVDPSWYPGNDVVDIVSADIYADAGDHSPQEETFASLQSLTGDTKLVALGEVGNIPDPASTGGVADWAYWVTWNGDFIKGEDYNPLEYKKEVFSAENIITRDEVDV

SEQ ID NO: 8 - protein, 327 aa, Myrothecium roridum
GTIENRQWLTYNPVDSAATTEARALLRYIQSQYGWRYLSGQQERAEVQWLKSNIGKTPAIQGSDLIDYSPSRVSYGATSTAVEDAIAFDRQGGIVTFTWHWNAPNCLYNSADQPWYFGFYTKATCFNIQAALAQGSNGADYKLLIRDIDAIAVQLKRLRDAKVPILFRPLHEPDGAWFWWGAKGSGPFKQLWDILYDRLTKYHGLHNMLWVCNTEKSDWYPGNNKCDIATTDVYVNAGDHSVQKSHWDALYGVSGGQRILALGEVGVIPDPERQASENVPWAYWMTWNGYFIRDGNYNSRNFLQSTFSNARVVTLDGTSPLGNWKSS

SEQ ID NO: 9 - protein, 452 aa, Chaetomium brasiliense
VPCGGGSNSGPRTYEAEDADLTGTNIDTAQSGFTGSGYVTGFDQATDKVTFKVDSPSLKLYDLSIRVAAIYGEKRTNVVLNNGASSEVYFAASETFTTVAAGQVLLNEGANTIDLVSNWGWYLIDSITLTPSTQRPPHNINPSPVNPSANADAKGLYTYLRSIYGKKILSGQQELSWSNWITTQTGKTPALVSVDLMDYSPSRVERGTVGTAVEEAITHAQRGGIVSVLWHWNAPTGLYDTEENKWWSGFYTRATDFDVAAALSSTTNANYTLILRDIDAIAVQLKKLQDAGVPVLFRPLHEAEGGWFWWGAKGAEPCKKLYALLYDRLTNYHKINNLIWVWNSILEEWYPGDATVDILSADVYAQGNGPISTQYNQLIELGKDKKMIAAAEVGAAPLPNLLQAYEAHWLWFTVWGDTFINNAEWNSVDVLKQVYTSDYVLTLDEIQGWRGA

SEQ ID NO: 10 - protein, 541 aa, Ascobolus stictoideus
QTYTLEAEAGTLTGVTVMNEIAGFSGTGYVGGWDEDADTVSLTFTSDATKLYDVKIRYSGPYGSKYTRISYNGATGGDISLPETTEWATVNAGQALLNAGSNTIKLHNNWGWYLIDAVILTPSVPRPPHQVTDALVNTNSNAVTKQLMKFLVSKYHKAYITGQQELHAHQWVEKNVGKSPAILGLDFMDYSPSRVEFGTTSQAVEQAIDFDKRGGIVTFAWHWNAPSGLINTPGSEWWRGFYTEHTTFDVAAALQNTTNANYNLLIRDIDAIAVQLKRLQTAGVPVLWRPLHEAEGGWFWWGAKGPEPAKKLYKILYDRLTNYHKLNNLIWVWNSVAKDWYPGDEIVDVLSFDSYPAQPGDHGPVSAQYNALVELGKDKKLIAATEVGTIPDPDLMQLYESYWSFFVTWEGEFIENGVHNSLEFLKKLYNNSFVLNLDTIQGWKNGAGSSTTTVKSTTTTPTTTIKSTTTTPVTTPTTVKTTTTPTTTATTVKSTTTTAGPTPTAVAGRWQQCGGIGFTGPTTCEAGTTCNVLNPYYSQCL

SEQ ID NO: 11 - protein, 526 aa, Chaetomium virescens
PRDPGATARTFEAEDATLAGTNVDTALSGFTGTGYVTGFDQAADKVTFTVDSASTELYDLSIRVAAIYGDKRTSVVLNGGASSEVYFPAGETWTNVAAGQLLLNQGSNTIDIVSNWGWYLIDSITLTPSTPRPAHQINEAPVNAAADKNAKALYSYLRSIYGKKILSGQQELSLSNWIAQQTGKTPALVSVDLMDYSPSRVERGTVGTAVEEAIQHHNRGGIVSVLWHWNAPTGLYDTEEHRWWSGFYTSATDFDVAAALSSTTNANYTLLIRDIDAIAVQLKRLQSAGVPVLFRPLHEAEGGWFWWGAKGPEPAKKLWGILYDRVTNHHQINNLLWVWNSILPEWYPGDATVDILSADVYAQGNGPMSTQYNQLIELGKDKKMIAAAEVGAAPLPDLLQAYEAHWLWFTVWGDSFINNADWNSLDTLKKVYTSDYVLTLDEIQGWQGSTPSATTTSSTTTPSATTTTTTPSTTATTATPSATTTASPVTYAEHWGQCAGKGWTGPTTCRPPYTCKYQNDWYSQCL

SEQ ID NO: 12 - protein, 527 aa, Paenibacillus ihumii
SSALPDTVVKEAPSASPTNGITVTFADAVLTGYGIEKRGSVKENEDTLYDGKGYISYFFDEDANAAEPVGSATFTVDVAEAGLYKLSLGYYLPEGYGDKVTSIEINGAGTGELTLDEPAAGTVRAEKMVSKVLLNAGSNTIKIMRGWGYYGIEHIKLEPAGAASSSNKLAAEDGPMTGALNNPEATPEARALMDYLLSQYGQKIISGQQTIEDIEWIKQQTGKYPAIFSTDLMDYSPSRIENGASSTEVEKMIEWYKRGGIVSLCWHWNAPKGIGGNEPGHEWWRGFYTEFTTFDVEFALNHLDSEDYQLLIRDIDAIAVQLKRLQDANVPVLWRPLHEAEGGWFWWGAKGPEPAKQLYRLMYDRLTHDHNLNNLIWIWNSEKKDWYPGDDVVDIVSVDIYNPAEDYNPSIAKYEGLVSLVNGKKMAALAENGPIPDPDALQAYGAEWSFFSTWTGDYIRDGKTNTMEHLKKVYHHDYVITLDELPADLYANPEFEAENGESAGMTRANGQESHSKGGYTTGMEPKN

SEQ ID NO: 13 - protein, 491 aa, Paenibacillus sp.
AITVPGFVVEPHTSSDQNQAIIATYNDASIEGYGIKKRDETTAKAEDDLYDGTGYISYFFEEDEKATAQKGSATFHVKAPENGLYELSLGYYIPEGNGDKATSIQVNGSGAGELMLSAPKQGTVRAEKKMTKVLLNSGNNSIQILRGWGYYGIEYIKLERVEPRITTQKTKMDPLSNSKASPQAKALMKFMTNQYGKKIISGQQTLEDATWIYQQTGKYPALVSSDLMDYSPSRVENGSTSNEVEKMMEWYKRGGIVSLSWHWNAPKGIGGNEPGHEWWRGFNTEFTTFDVEYALDHPESEDYKLLIRDIDAIAAQLKRLQEHHIPVLWRPLHEAEGGWFWWGAKGPEPAKKLYRLMYERLTEKHKLNNLIWVWNSVKEEWYPGDDVVDMVSVDIYNPPGDHSPSIAKYDELLFLSKHKKLVALAENGPIPDPDLLQTYGAHWSYFNTWTGDVLRDGKTNTKEHLKKVYNHDNVITLDELPKGLYGCPRWK

SEQ ID NO: 14 - protein, 458 aa, Salipaludibacillus agaradhaerens
NYESEVRRFEAEDATLNGVTVKNSEPGFSGTGYVGDFEDSSQSVTFHVDVPETDLYTLTIGYGAIYGSEKVANVLVNGEKLSSFTMGSGFGKASAGNIVLNSGSNTISITPDWTHFAIDYIEVKLTPEPIKHNVEKKLINPNATDEAKVLMSYLVDNFGEKILSGQHDFPNTRPDDLEYIYEITGKYPAILGLDFIDNSPSRVEYGAFADETPVAINWWNKGGIVTFTWHWNAPKDLLDEPGNEWWRGFYTEATTFDVEYALNHPDSEDYKLLIRDIDVIADELKKLQKADVPVLWRPLHEAEGKWFWWGKKGPEPAKELWLLMYDRMTNYHNLNNLIWVWNSIEEDWYPGDEYVDIVSFDSYPGDYNYSPMSGQYEALKELSSNKKIIAIAENGPIPDPDLLQRYHAHYSWFTTWNGDILREQNSEEHLKNVYNHDYVITLDELPDFETYKEDVPLE

SEQ ID NO: 15 - protein, 370 aa, Geobacillus tepidamans
KKQKNPSKPNSKRVENLVDPLATDDTKSLFAYLKDVRGKQVLFGHQHAIDEGLTLIGSKELESEVKNSVGDFPAVFGWDTLSLEGKEKPGVPNDPKQSRANLVASMKKVHKLGGIIALSAHMPNFVTGGSFNDTTGNVVEHILPGGDKNAEFNSFLDNIAQFAKELKDDKGKQIPILFRPFHEQNGSWFWWGAKTTTPSQYIEIYRYTVEYLRDKKGVHNFLYVYSPNGTFGGSEANYLTTYPGDDYVDILGMDQYDNQSNPGTTQFLTNLVKDLEMISKLADTKGKIAAFSEFGYSPQGMKTTGNGDLKWFTKVLNAIKADRNAKRIAYMQTWANFGLNGNLFVPYNDAPNGLGDHELLPDFINYYKDP

SEQ ID NO: 16 - protein, 1062 aa, Bacillus sp. SWT81
SQEGRQLNMADEDASKYTKELFAFLQDVSGSQVLFGQQHATDEGLTLTNPAPRTGSTQSEVFNAVGDYPAVFGWDTNSLDGREKPGIAGNVEQSIKNTAQSMKVAHDLGGIITLSMHPDNFVTGGPYGDTTGNVVKEILPGGSKHAEFNAWLDNIAALAHELKDENGEPIPMIFRPFHEQTGSWFWWGASTTSPEQYKAIFRYTVEYLRDVKGVNNILYGFSPGAGPAGDVNRYLETYPGDDYVDIFGIDNYDNKDNAGSEAWLSGMVKDLAMISRLAEQKEKVAAFTEYGYSATGINRQGNTLDWYTRVLDAIAADEDARKISYMLTWANFGWPNNMYVPYRDIHNELGGDHELLPDFEAFHADDYTAFRDEIKGKIYNTGKEYTVSPHEPFMYVISPITGSTVTSETVTIQAKVANDEHARVTFRVDGSSLEEEMVFNDDTLYYTGSFTPDAAVNGGAVDVIVAYYSSGEKVQEETIRLFVKIPEMSLLTLTFDDDINGIKSNGTWPEDGVTSEIDHAIVDGDGKLMFSVQGMSPTETWQELKLELTELSDVNIDAVKKMKFDALIPAGSEEGSVQGIVQLPPDWETKYGMNETTKSIKDLETVTVNGSDYKRLEVTVSIDNQGGATGIALSLVGSQLDLLEPVYIDNIELLNSFEAPPADSFLVDDFEGYFGDDTLLHRNYSSNGDPITLSLTSEFKNNGEFGLKYDYSIGSMGYAGRQTSLGPVDWSGANAFEFWMKHGQLEGNHLTVQIRIGDVSFEKNLELMDAHEGVVTIPFSEFAPAAWENKPGVIIDEQKLKRVSQFALYTGGARQSGTIYFDDLRAVYDESLPSVPVPKEEEEEKEVAPIIYHFESGIDNWEGGQATHSNGHLKVTVRLGEGQQTEVKKTSNYNLTGYNYIVANIKHDDTGMFGSDPLQVKIFTKAGGWVWADSGNQPIYSDDYTQVVYDITTLANKNAVQEIGFEFLAPSGSSGTTNPFIDSVAIVTSLDQLSEQPEQPEQPGTPDTDDNKEDKDRRNVEVNEEGQKLPKTATSIFNYLLIGFVFVGIGFSLFIYKRRKTV

SEQ ID NO: 17 - protein, 309 aa, Bacillus bogoriensis
ANSGFYVSGTTLYDANGNPFVMRGINHGHAWYKDQATTAIEGIANTGANTVRIVLSDGGQWTKDDIHTVRNLISLAEDNHLVAVPEVHDATGYDSIASLNRAVDYWIEMRSALIGKEDTVIINIANEWFGSWEGDAWADGYKQAIPRLRNAGLNHTLMVDAAGWGQFPQSIHDYGREVFNADPQRNTMFSIHMYEYAGGNASQVRTNIDRVLNQDLALVIGEFGHRHTNGDVDEATIMSYSEQRGVGWLAWSWKGNGPEWEYLDLSNDWAGNNLTAWGNTIVNGPYGLRETSRLSTVFTGGGSDGGTSP

SEQ ID NO: 18 - protein, 309 aa, Artificial Sequence
  Synthetic Construct
ANSGFYVSGTTLYDANGNPFVMRGINHGHTWYKDQATTAIEGIANTGANTVRIVLSDGGQWTKDDIHTVRNLISLAEDNHLVAVLEVHDATGQDDIASLNRAVDYWIEMRSALIGKEKTVIINIANEWFGSWEGDPWARGYKQAIPRLRNAGLNHTLMVDAAGWGQFPQSIHDYGREVFNADPQRNTMFSIHMYEYAGGTARQVRTNIDGVLNQDLALVIGEFGHRHTNGDVDEATIMSYSEQRGVGWLAWSWKGNGPEFEYLDLSNDWAGNNLTAWGNTIVHGPYGIRETSRPVTVFTGGGSDGGTSP

SEQ ID NO: 19 - protein, 299 aa, Bacillus lentus
ASGFYVSGTILCDSTGNPFKIRGINHAHSWFKNDSATAMEAIAATGANTVRIVLSNGQQYAKDDANTVSNLLSLANQHKLIAILEVHDATGSDSVSALDHAVDYWIEMKNVLVGKEDRVLINIANEWYGTWDSNGWADGYKSAIPKLRNAGINHTLIVDAAGWGQYPQSIVDKGNEVFNSDPLRNTIFSIHMYEYAGGNADMVRANIDQVLNKGLAVIIGEFGHYHTGGDVDETAIMSYTQQKGVGWLAWSWKGNGAEWLYLDLSYDWAGNHLTEWGETIVNGANGLKATSTRAPIFGN

SEQ ID NO: 20 - protein, 297 aa, Paenibacillus sp.A1
MATGFYVSGNKLYDSTGKPFVMRGVNHGHSWFKNDLNTAIPAIAKTGANTVRIVLSNGSLYTKDDLNAVKNIINVVNQNKMIAVLEVHDATGKDDYNSLDAAVNYWISIKEALIGKEDRVIVNIANEWYGTWNGSAWADGYKKAIPKLRNAGIKNTLIVDAAGWGQFPQSIVDYGQSVFAADSQKNTVFSIHMYEYAGKDAATVKANMENVLNKGLALIIGEFGGYHTNGDVDEYAIMRYGQEKGVGWLAWSWYGNSSGLNYLDMATGPNGSLTSFGNTVVNDTYGIKNTSQKAGIF

SEQ ID NO: 21 - protein, 298 aa, Artificial Sequence
  Synthetic Construct
MATGFYVSGNKLYDSTGKEFVMRGVNHGHTWFKNDLNEAIPAIAKTGANTVRIVLSNGVQYTRDDLDAVKNIINVVNQNKMIAVLEVHDATGKDDYDSLDAAINYWISIKEALIGKEDRVIVNIANEWMGTWNGSAWADGYKKAIPKLRNAGIKNTLIVDAAGWGQYPQSIVDYGQSVFAADSLKNTVFSIHMYEYAGKDAATVKANMENVLNKGLALIIGEFGCYHVNGDVDELAIMRYGQELGVGWLAWSWYGNSDGLRYLDMATGPNGSLTSFGNTVVNDTYGIKNTSQKAGIFQ

SEQ ID NO: 22 - protein, 298 aa, Artificial sequence
  Synthetic Construct
MATGFYVSGNKLYDSTGKEFVMRGVNHGHTWFKNDLNEAIPAIAKTGANTVRIVLSNGVQYTRDDLNAVKNIINVVNQNKMIAVLEVHDATGKDDYDSLDAAVNYWISIKEALIGKEDRVIVNIANEWMGTWNGSAWADGYKKAIPKLRNAGIKNTLIVDAAGWGQFSQSIVDYGQSVFAADSLKNTVFSIHMYEYAGKDAATVKANMENVLNKGLALIIGEFGCYHVNGDVDELAIMRYGQELGVGWLAWSWYGNSDGLRYLDMATGPNGSLTSFGNTVVNDTYGIKNTSQKAGIFQ

SEQ ID NO: 23 - protein, 298 aa, Artificial Sequence
  Synthetic Construct
MATGFYVSGTKLYDSTGKEFVMRGVNHGHTWFKNDLNEAIPAIAKTGANTVRIVLSNGVQYTRDDLDAVKNIINVVNQNKMIAVLEVHDATGKDDYDSLDAAVNYWISIKEALIGKEDRVIVNIANEWMGTWNGSAWADGYKQAIPKLRNAGIKNTLIVDAAGWGQFSQSIVDYGQSVFAADSLKNTVFSIHMYEYAGKDAATVKANMENVLNKGLALIIGEFGPYHVNGDVDELAIMRYGQELGVGWLAWSWYGNSDGLRYLDMATGPNGSLTSFGNTVVNDTYGIKNTSQKAGIFQ